European Patent Specification EP 4 271 702 B1, published November 6, 2024. Title: Chlorotoxin derivatives and use thereof. Applicant: Vascular Venture Korlátolt Felelõsségû Társaság. The sequence listing filed with the application follows.

SEQUENCE LISTING (44 sequences)

SEQ ID NO: 1 - protein, 36 aa, Leiurus quinquestriatus
MCMPCFTTDHQMARKCDDCCGGKGRGKCYGPQCLCR

SEQ ID NO: 2 - protein, 36 aa, Artificial Sequence
  monolysine (K27) mutant of CTX
MCMPCFTTDHQMARRCDDCCGGRGRGKCYGPQCLCR

SEQ ID NO: 3 - protein, 36 aa, Artificial Sequence
  Chlorotoxin derivative
AMCMPCFTTDHQTARRCDKCCGGYGRCFGYQCLCNR

SEQ ID NO: 4 - protein, 38 aa, Artificial Sequence
  Chlorotoxin derivative
AMCMPCFTTDHQTARRCDKCCGGYGRCFGYQCLCNRGY

SEQ ID NO: 5 - protein, 37 aa, Artificial Sequence
  Chlorotoxin derivative
AMCMPCFTTDHQTARRCDKCCGGYGRCFGYQCLCNRG

SEQ ID NO: 6 - protein, 37 aa, Artificial Sequence
  Chlorotoxin derivative
MCMPCFTTDHQTARRCDKCCGGYGRCFGYQCLCNRGY

SEQ ID NO: 7 - protein, 36 aa, Artificial Sequence; identical to SEQ ID NO: 3
  Chlorotoxin derivative

SEQ ID NO: 8 - protein, 36 aa, Artificial Sequence
  Chlorotoxin derivative
CMPCFTTDHQTARRCDKCCGGYGRCFGYQCLCNRGY

SEQ ID NO: 9 - protein, 35 aa, Artificial Sequence
  Chlorotoxin derivative
AMCMPCFTTDHQTARRCDKCCGGYGRCFGYQCLCN

SEQ ID NO: 10 - protein, 38 aa, Artificial Sequence
  Chlorotoxin derivative
AMCMPCFTTDHQTARRCRDCCGGYGKCFGYQCLCNRGY

SEQ ID NO: 11 - protein, 38 aa, Artificial Sequence
  Chlorotoxin derivative
AMCMPCFTTDHQTARRCIKCCGGYGYCFGYQCLCNRGY

SEQ ID NO: 12 - protein, 38 aa, Artificial Sequence
  Chlorotoxin derivative
AMCMPCFTTDHQTARRCHKCCGGYGWCFGYQCLCNRGY

SEQ ID NO: 13 - protein, 38 aa, Artificial Sequence
  Chlorotoxin derivative
AMCMPCFTTDHQTARRCDRCCGGYGKCFGYQCLCNRGY

SEQ ID NO: 14 - protein, 38 aa, Artificial Sequence
  Chlorotoxin derivative
AMCMPCFTTDHQTARRCLKCCGGYGQCFGYQCLCNRGY

SEQ ID NO: 15 - protein, 35 aa, Artificial Sequence
  Chlorotoxin derivative
AMCMPCFTTDHQTARRCDKCCGGYGRCFGYQCLCR

SEQ ID NO: 16 - protein, 38 aa, Artificial Sequence
  Chlorotoxin derivative
AMCMPCFTTDHQTARRCKDCCGGYGRCFGYQCLCNRGY

SEQ ID NO: 17 - protein, 38 aa, Artificial Sequence
  Chlorotoxin derivative
AMCMPCFTTDHQTARRCKKCCGGYGKCFGYQCLCNRGY

SEQ ID NO: 18 - protein, 37 aa, Artificial Sequence
  Chlorotoxin derivative
MCMPCFTTDHQTARRCKKCCGGYGKCFGYQCLCNRGY

SEQ ID NO: 19 - protein, 38 aa, Artificial Sequence
  Chlorotoxin derivative
AMCMPCFTTDHQTARRCKWCCGGYGICFGYQCLCNRGY

SEQ ID NO: 20 - protein, 38 aa, Artificial Sequence
  Chlorotoxin derivative
AMCMPCFTTDHQTARRCVKCCGGYGFCFGYQCLCNRGY

SEQ ID NO: 21 - protein, 38 aa, Artificial Sequence
  Chlorotoxin derivative
AMCMPCFTTDHQTARRCKHCCGGYGVCFGYQCLCNRGY

SEQ ID NO: 22 - protein, 38 aa, Artificial Sequence
  Chlorotoxin derivative
AMCMPCFTTDHQTARRCKFCCGGYGRCFGYQCLCNRGY

SEQ ID NO: 23 - protein, 38 aa, Artificial Sequence
  Chlorotoxin derivative
AMCMPCFTTDHQTARRCKWCCGGYGWCFGYQCLCNRGY

SEQ ID NO: 24 - protein, 34 aa, Artificial Sequence
  Chlorotoxin derivative
AMCMPCFTTDHQTARRCDKCCGGYGRCFGYQCLC

SEQ ID NO: 25 - protein, 38 aa, Artificial Sequence
  Chlorotoxin derivative
AMCMPCFTTDHQTARRCKSCCGGYGFCFGYQCLCNRGY

SEQ ID NO: 26 - protein, 38 aa, Artificial Sequence
  Chlorotoxin derivative
AMCMPCFTTDHQTARRCKRCCGGYGRCFGYQCLCNRGY

SEQ ID NO: 27 - protein, 38 aa, Artificial Sequence
  Chlorotoxin derivative
AMCMPCFTTDHQTARRCRFCCGGYGKCFGYQCLCNRGY

SEQ ID NO: 28 - protein, 38 aa, Artificial Sequence
  Chlorotoxin derivative
AMCMPCFTTDHQTARRCVWCCGGYGKCFGYQCLCNRGY

SEQ ID NO: 29 - protein, 38 aa, Artificial Sequence
  Chlorotoxin derivative
AMCMPCFTTDHQTARRCDDCCGGYGKCFGYQCLCNRGY

SEQ ID NO: 30 - protein, 38 aa, Artificial Sequence
  Chlorotoxin derivative
AMCMPCFTTDHQTARRCRKCCGGYGRCFGYQCLCNRGY

SEQ ID NO: 31 - protein, 38 aa, Artificial Sequence
  Chlorotoxin derivative
AMCMPCFTTDHQTARRCWKCCGGYGWCFGYQCLCNRGY

SEQ ID NO: 32 - protein, 38 aa, Artificial Sequence
  Chlorotoxin derivative
AMCMPCFTTDHQTARRCRRCCGGYGKCFGYQCLCNRGY

SEQ ID NO: 33 - protein, 38 aa, Artificial Sequence
  Chlorotoxin derivative
AMCMPCFTTDHQTARRCRWCCGGYGKCFGYQCLCNRGY

SEQ ID NO: 34 - protein, 38 aa, Artificial Sequence
  Chlorotoxin derivative
AMCMPCFTTDHQTARRCLKCCGGYGSCFGYQCLCNRGY

SEQ ID NO: 35 - protein, 38 aa, Artificial Sequence
  Chlorotoxin derivative
  misc_feature (1)..(2): Xaa can be any naturally occurring amino acid
  misc_feature (18)..(19): Xaa can be any naturally occurring amino acid
  misc_feature (26)..(26): Xaa can be any naturally occurring amino acid
  misc_feature (35)..(38): Xaa can be any naturally occurring amino acid
XXCMPCFTTDHQTARRCXXCCGGYGXCFGYQCLCXXXX

SEQ ID NO: 36 - protein, 38 aa, Artificial Sequence
  Chlorotoxin derivative
AMCMPCSSSDHESARRCDKCCGGYGRCFGYQCLCNRGY

SEQ ID NO: 37 - protein, 38 aa, Artificial Sequence
  Chlorotoxin derivative
AMCMPCFTTDHQTARRCDKCCGGYGRCFGYQCLCNRRR

SEQ ID NO: 38 - protein, 38 aa, Artificial Sequence
  Chlorotoxin derivative
AMCMPCSSSDHESARRCDKCCGGYGRCFGYQCLCNRRR

SEQ ID NO: 39 - protein, 38 aa, Artificial Sequence
  Chlorotoxin derivative
AMCMPCSSSDHQTARRCDKCCGGYGRCFGYQCLCNRGY

SEQ ID NO: 40 - protein, 38 aa, Artificial Sequence
  Chlorotoxin derivative
AMCMPCSSSDHESARRCRDCCGGYGKCFGYQCLCNRGY

SEQ ID NO: 41 - protein, 38 aa, Artificial Sequence
  Chlorotoxin derivative
AMCMPCFTTDHQTARRCRDCCGGYGKCFGYQCLCNRRR

SEQ ID NO: 42 - protein, 38 aa, Artificial Sequence
  Chlorotoxin derivative
AMCMPCSSSDHESARRCRDCCGGYGKCFGYQCLCNRRR

SEQ ID NO: 43 - protein, 38 aa, Artificial Sequence
  Chlorotoxin derivative
  misc_feature (1)..(2): Xaa can be any naturally occurring amino acid
  misc_feature (7)..(9): Xaa can be any naturally occurring amino acid
  misc_feature (12)..(13): Xaa can be any naturally occurring amino acid
  misc_feature (18)..(19): Xaa can be any naturally occurring amino acid
  misc_feature (26)..(26): Xaa can be any naturally occurring amino acid
  misc_feature (35)..(38): Xaa can be any naturally occurring amino acid
XXCMPCXXXDHXXARRCXXCCGGYGXCFGYQCLCXXXX

SEQ ID NO: 44 - protein, 645 aa, Artificial Sequence
  CTXD8-CAR construct
MLLLVTSLLLCELPHPAFLLIPAMCMPCSSSDHESARRCRDCCGGYGKCFGYQCLCNRRRTTTPAPRPPTPAPTIASQPLSLRPEACRPAAGGAVHTRGLDFACDMFWVLVVVGGVLACYSLLVTVAFIIFWVRSKRSRGGHSDYMNMTPRRPGPTRKHYQPYAPPRDFAAYRSGGGRVKFSRSADAPAYQQGQNQLYNELNLGRREEYDVLDKRRGRDPEMGGKPQRRKNPQEGLYNELQKDKMAEAYSEIGMKGERRRGKGHDGLYQGLSTATKDTYDALHMQALPPRASRAEGRGSLLTCGDVEENPGPMPPPRLLFFLLFLTPMEVRPEEPLVVKVEEGDNAVLQCLKGTSDGPTQQLTWSRESPLKPFLKLSLGLPGLGIHMRPLAIWLFIFNVSQQMGGFYLCQPGPPSEKAWQPGWTVNVEGSGELFRWNVSDLGGLGCGLKNRSSEGPSSPSGKLMSPKLYVWAKDRPEIWEGEPPCLPPRDSLNQSLSQDLTMAPGSTLWLSCGVPPDSVSRGPLSWTHVHPKGPKSLLSLELKDDRPARDMWVMETGLLLPRATAQDAGKYYCHRGNLTMSFHLEITARPVLWHWLLRTGGWKVSAVTLAYLIFCLCSLVGILHLQRALVLRRKRKRMTDPTRRF